European Patent Application EP 4 800 031 A2, published September 2, 2026. Title: TSLP-Binding Molecules, IL-33-Binding Molecules, and Bispecific Antigen-Binding Molecules, and Uses Thereof. Applicant: NEWSOARA BIOPHARMACEUTICAL TECHNOLOGY (SUZHOU) CO., LTD. The sequence listing filed with the application follows.

SEQUENCE LISTING (218 sequences)

SEQ ID NO: 1 - protein, 10 aa, synthetic construct
GSNFSLYAMS

SEQ ID NO: 2 - protein, 9 aa, synthetic construct
RIRDNGRTN

SEQ ID NO: 3 - protein, 7 aa, synthetic construct
DNRVTTF

SEQ ID NO: 4 - protein, 115 aa, synthetic construct
QVQLVESGGGLVQPGGSLTLSCVAAGSNFSLYAMSYYRQVPGKQRELVARIRDNGRTNYADSVKDRFTISRDSAKNTVYLQMHSLKPEDTAVYYCNADNRVTTFWGRGTQVTVSS

SEQ ID NO: 5 - protein, 10 aa, synthetic construct
GSIFSIDAMG

SEQ ID NO: 6 - protein, 7 aa, synthetic construct
AIGSGTY

SEQ ID NO: 7 - protein, 8 aa, synthetic construct
GDSYPDEY

SEQ ID NO: 8 - protein, 115 aa, synthetic construct
QLQLVESGGGLVQPGGSLRLSCAASGSIFSIDAMGWYRQAPGKERELVAAIGSGTYYADSVKGRFTISRDNAKKNTLYLQMDSLKPEDTAIYYCASGDSYPDEYWGQGTQVTVSA

SEQ ID NO: 9 - protein, 10 aa, synthetic construct
ESDFSIYIMG

SEQ ID NO: 10 - protein, 9 aa, synthetic construct
TITPGGNTN

SEQ ID NO: 11 - protein, 9 aa, synthetic construct
RNIFRNVDY

SEQ ID NO: 12 - protein, 117 aa, synthetic construct
QLQLVESGGGLVQPGGSLRLSCAASESDFSIYIMGWYRQAPGKQRELVVTITPGGNTNYVDSVKGRFTISRDNTMNTAYLQMNSLKPDDTAVYYCNARNIFRNVDYSGKGTLVTVSS

SEQ ID NO: 13 - protein, 10 aa, synthetic construct
GIEFSIYIMG

SEQ ID NO: 14 - protein, 9 aa, synthetic construct
TVTPGGNTN

SEQ ID NO: 15 - protein, 9 aa, synthetic construct
RNIFRNMDY

SEQ ID NO: 16 - protein, 117 aa, synthetic construct
QVQLVESGGGLVQPGGSLRLSCVASGIEFSIYIMGWYRQAPGKQRELVATVTPGGNTNYADSVKGRFTISRDNTKNTAYLQMNSLKPDDTAVYYCNARNIFRNMDYQGKGTLVTVSS

SEQ ID NO: 17 - protein, 10 aa, synthetic construct
GSDFNIYIMG

SEQ ID NO: 18 - protein, 9 aa, synthetic construct
TITPGGNTN

SEQ ID NO: 19 - protein, 9 aa, synthetic construct
RNIFRYMDY

SEQ ID NO: 20 - protein, 117 aa, synthetic construct
QVQLVESGGGSVQPGGSLRLSCAASGSDFNIYIMGWYQQAPGKQRELVATITPGGNTNYVDSVKGRFTISRDNTKNTAYLQMNSLKPDDTAVYYCNARNIFRYMDYWGKGTLVTVSS

SEQ ID NO: 21 - protein, 10 aa, synthetic construct
GFIFDDYAIA

SEQ ID NO: 22 - protein, 10 aa, synthetic construct
FISNSDGTAY

SEQ ID NO: 23 - protein, 23 aa, synthetic construct
EGRMGTHSRDSVYFWAFSALYDY

SEQ ID NO: 24 - protein, 132 aa, synthetic construct
QVQLVESGGGLVQAGGSLRLSCAASGFIFDDYAIAWFRQAPGKEREGVSFISNSDGTAYYADSVKGRFTISSDNAKNTVYLQMDSLKPDDTADYYCAAEGRMGTHSRDSVYFWAFSALYDYWGQGTQVTVSS

SEQ ID NO: 25 - protein, 10 aa, synthetic construct
GFTFDDYAIT

SEQ ID NO: 26 - protein, 10 aa, synthetic construct
YISNSDGMTY

SEQ ID NO: 27 - protein, 23 aa, synthetic construct
EGIMGTHNRDNVYFWAFSALYDY

SEQ ID NO: 28 - protein, 132 aa, synthetic construct
QLQLVESGGGLVQAGGSLRLSCAASGFTFDDYAITWFRQAPGKEREGVAYISNSDGMTYYVDSVKGRFTISSDNAKNTVYLQMDSLKPEDTAVYYCAAEGIMGTHNRDNVYFWAFSALYDYWGQGTQVTVSS

SEQ ID NO: 29 - protein, 10 aa, synthetic construct
GFTFDDYAIT

SEQ ID NO: 30 - protein, 10 aa, synthetic construct
YISNFDGMTY

SEQ ID NO: 31 - protein, 23 aa, synthetic construct
EGRMGTHSRDSVYFWAFSALYDH

SEQ ID NO: 32 - protein, 132 aa, synthetic construct
QVQLVESGGGLVQAGGSLRLSCAASGFTFDDYAITWFRQAPGKEREGVAYISNFDGMTYYADSVKGRFTISSDNAKNTVYLQMDSLKPEDTAVYYCAAEGRMGTHSRDSVYFWAFSALYDHWGQGTQVTVSS

SEQ ID NO: 33 - protein, 10 aa, synthetic construct
GFTFDDYAIT

SEQ ID NO: 34 - protein, 10 aa, synthetic construct
YISNSDGMTY

SEQ ID NO: 35 - protein, 23 aa, synthetic construct
EGRMGTHSRDSVYFWAFSALYDY

SEQ ID NO: 36 - protein, 132 aa, synthetic construct
QVQLVESGGGLVQAGGSLRLSCAASGFTFDDYAITWFRQAPGKEREGVAYISNSDGMTYYADSVKGRFTISSDNAKNTVYLQMDSLKPEDTAVYYCAAEGRMGTHSRDSVYFWAFSALYDYWGQGTQVTVSS

SEQ ID NO: 37 - protein, 10 aa, synthetic construct
GFTFDDYAIT

SEQ ID NO: 38 - protein, 10 aa, synthetic construct
YISNNDGMTY

SEQ ID NO: 39 - protein, 23 aa, synthetic construct
EGRMGTHSRDSVYFWAFSALYDY

SEQ ID NO: 40 - protein, 132 aa, synthetic construct
QVQLVESGGGLVQAGGSLRLSCAASGFTFDDYAITWFRQAPGKEREGVAYISNNDGMTYYADSVKGRFTISSDNAKNPVYLQMDSLKPEDTAVYYCAAEGRMGTHSRDSVYFWAFSALYDYWGQGTQVTVSS

SEQ ID NO: 41 - protein, 10 aa, synthetic construct
GFTFGDYAIT

SEQ ID NO: 42 - protein, 10 aa, synthetic construct
YISNFDGMTY

SEQ ID NO: 43 - protein, 23 aa, synthetic construct
EGRMGTHSRDSVYFWAFSALYDY

SEQ ID NO: 44 - protein, 132 aa, synthetic construct
QVQLVESGGGLVQAGGSLRLSCAASGFTFGDYAITWFRQAPGKEREGVAYISNFDGMTYYADSVKGRFTISSDNAKNTVYLQMDSLKPEDTAVYYCAAEGRMGTHSRDSVYFWAFSALYDYWGQGTQVTVSS

SEQ ID NO: 45 - protein, 10 aa, synthetic construct
GFIFDDYAIA

SEQ ID NO: 46 - protein, 10 aa, synthetic construct
FISNSDGTAY

SEQ ID NO: 47 - protein, 23 aa, synthetic construct
EGRMGTHSGDSVYFWSFSALYDY

SEQ ID NO: 48 - protein, 132 aa, synthetic construct
QVQLVESGGGLVQAGGSLRLSCAASGFIFDDYAIAWFRQAPGKEREGVSFISNSDGTAYYADSVKGRFTISSDNAKNTVYLQMDSLKPDDTADYYCAAEGRMGTHSGDSVYFWSFSALYDYWGQGTQVTVSS

SEQ ID NO: 49 - protein, 10 aa, synthetic construct
GFNFDDYAIA

SEQ ID NO: 50 - protein, 10 aa, synthetic construct
FISNSDGTAY

SEQ ID NO: 51 - protein, 23 aa, synthetic construct
EGRMGTHSRDSVYFWSFSALYDY

SEQ ID NO: 52 - protein, 132 aa, synthetic construct
QLQLVESGGGLVQAGGSLRLSCAASGFNFDDYAIAWFRQAPGKEREGVSFISNSDGTAYYADSVKGRFTISSDNAKNTVYLQMDSLKPDDTADYYCAAEGRMGTHSRDSVYFWSFSALYDYWGQGTQVTVSS

SEQ ID NO: 53 - protein, 10 aa, synthetic construct
GFSFDDYAIA

SEQ ID NO: 54 - protein, 10 aa, synthetic construct
FISNSDGTAY

SEQ ID NO: 55 - protein, 23 aa, synthetic construct
EGRMGTHSRDSVYFWSFSALYDY

SEQ ID NO: 56 - protein, 132 aa, synthetic construct
QVQLVESGGGLVQAGGSLRLSCAASGFSFDDYAIAWFRQAPGKEREGVSFISNSDGTAYYADSVKGRFTISSDNAKNTVYLQMDSLKPDDTADYYCAAEGRMGTHSRDSVYFWSFSALYDYWGQGTQVTVSS

SEQ ID NO: 57 - protein, 10 aa, synthetic construct
GGTFERLAMG

SEQ ID NO: 58 - protein, 10 aa, synthetic construct
FISNSDGTAY

SEQ ID NO: 59 - protein, 23 aa, synthetic construct
EGRMGTHSRDSVYFWSFSALYDY

SEQ ID NO: 60 - protein, 132 aa, synthetic construct
QLQLVESGGGLVQPGGSLRLSCVLSGGTFERLAMGWFRQAPGKEREGVSFISNSDGTAYYADSVKGRFTISSDNAKNTVYLQMDSLKPDDTADYYCAAEGRMGTHSRDSVYFWSFSALYDYWGQGTQVTVSA

SEQ ID NO: 61 - protein, 10 aa, synthetic construct
GFTFDDYAIT

SEQ ID NO: 62 - protein, 10 aa, synthetic construct
YISNNDHNTY

SEQ ID NO: 63 - protein, 23 aa, synthetic construct
EGRMGTHSRESSYFWTFPALYDY

SEQ ID NO: 64 - protein, 132 aa, synthetic construct
QVQLVESGGGLVQAGGSLRLSCAASGFTFDDYAITWFRQAPGKEREGVSYISNNDHNTYYADSVKGRFTISSDNAKNTVYLQMDSLKPEDTAVYYCAAEGRMGTHSRESSYFWTFPALYDYWGQGTQVTVSS

SEQ ID NO: 65 - protein, 132 aa, synthetic construct
QVQLLESGGGLVQPGGSLRLSCAASGFTFGDYAITWFRQAPGKGLEGVAYISNFDGMTYYADSVKGRFTISSDNSKNTVYLQMNSLRAEDTAVYYCAAEGRMGTHSRDSVYFWAFSALYDYWGQGTLVTVSS

SEQ ID NO: 66 - protein, 132 aa, synthetic construct
EVQLLESGGGLVQPGGSLRLSCAASGFTFGDYAITWFRQAPGKGLEGVAYISNFDGMTYYADSVKGRFTISSDNSKNTVYLQMNSLRAEDTAVYYCAAEGRMGTHSRDSVYFWAFSALYDYWGQGTLVTVSS

SEQ ID NO: 67 - protein, 132 aa, synthetic construct
QVQLLESGGGLVQPGGSLRLSCAASGFTFGDYAITWFRQAPGKGLEGVAYISNFDGMTYYADSVKGRFTISRDNSKNTVYLQMNSLRAEDTAVYYCAAEGRMGTHSRDSVYFWAFSALYDYWGQGTLVTVSS

SEQ ID NO: 68 - protein, 132 aa, synthetic construct
EVQLLESGGGLVQPGGSLRLSCAASGFTFGDYAITWFRQAPGKGLEGVAYISNFDGMTYYADSVKGRFTISRDNSKNTVYLQMNSLRAEDTAVYYCAAEGRMGTHSRDSVYFWAFSALYDYWGQGTLVTVSS

SEQ ID NO: 69 - protein, 132 aa, synthetic construct
EVQLLESGGGLVQAGGSLRLSCAASGFTFGDYAITWFRQAPGKGLEGVAYISNFDGMTYYADSVKGRFTISSDNSKNTVYLQMNSLRAEDTAVYYCAAEGRMGTHSRDSVYFWAFSALYDYWGQGTLVTVSS

SEQ ID NO: 70 - protein, 132 aa, synthetic construct
EVQLLESGGGLVQPGGSLRLSCAASGFTFGDYAITWFRQAPGKELEGVAYISNFDGMTYYADSVKGRFTISSDNSKNTVYLQMNSLRAEDTAVYYCAAEGRMGTHSRDSVYFWAFSALYDYWGQGTLVTVSS

SEQ ID NO: 71 - protein, 132 aa, synthetic construct
EVQLLESGGGLVQPGGSLRLSCAASGFTFGDYAITWFRQAPGKGREGVAYISNFDGMTYYADSVKGRFTISSDNSKNTVYLQMNSLRAEDTAVYYCAAEGRMGTHSRDSVYFWAFSALYDYWGQGTLVTVSS

SEQ ID NO: 72 - protein, 132 aa, synthetic construct
EVQLLESGGGLVQPGGSLRLSCAASGFTFGDYAITWFRQAPGKEREGVAYISNFDGMTYYADSVKGRFTISSDNSKNTVYLQMNSLRAEDTAVYYCAAEGRMGTHSRDSVYFWAFSALYDYWGQGTLVTVSS

SEQ ID NO: 73 - protein, 132 aa, synthetic construct
EVQLLESGGGLVQPGGSLRLSCAASGFTFGDYAITWFRQAPGKGLEGVAYISNFDGMTYYADSVKGRFTISSDNAKNTVYLQMNSLRAEDTAVYYCAAEGRMGTHSRDSVYFWAFSALYDYWGQGTLVTVSS

SEQ ID NO: 74 - protein, 132 aa, synthetic construct
EVQLLESGGGLVQPGGSLRLSCAASGFTFGDYAITWFRQAPGKGLEGVAYISNFDGMTYYADSVKGRFTISSDNSKNTVYLQMDSLRAEDTAVYYCAAEGRMGTHSRDSVYFWAFSALYDYWGQGTLVTVSS

SEQ ID NO: 75 - protein, 132 aa, synthetic construct
EVQLLESGGGLVQPGGSLRLSCAASGFTFGDYAITWFRQAPGKGLEGVAYISNFDGMTYYADSVKGRFTISSDNSKNTVYLQMNSLRPEDTAVYYCAAEGRMGTHSRDSVYFWAFSALYDYWGQGTLVTVSS

SEQ ID NO: 76 - protein, 132 aa, synthetic construct
EVQLLESGGGLVQPGGSLRLSCAASGFTFGDYAITWFRQAPGKGLEGVSYISNFDGMTYYADSVKGRFTISSDNSKNTVYLQMNSLRAEDTAVYYCAAEGRMGTHSRDSVYFWAFSALYDYWGQGTLVTVSS

SEQ ID NO: 77 - protein, 132 aa, synthetic construct
EVQLVESGGGLVQPGGSLRLSCAASGFTFGDYAITWFRQAPGKGLEGVAYISNFDGMTYYADSVKGRFTISSDNSKNTVYLQMNSLRAEDTAVYYCAAEGRMGTHSRDSVYFWAFSALYDYWGQGTLVTVSS

SEQ ID NO: 78 - protein, 132 aa, synthetic construct
EVQLLESGGGLVQPGGSLRLSCAASGFTFGDYAITWVRQAPGKGLEGVAYISNFDGMTYYADSVKGRFTISSDNSKNTVYLQMNSLRAEDTAVYYCAAEGRMGTHSRDSVYFWAFSALYDYWGQGTLVTVSS

SEQ ID NO: 79 - protein, 10 aa, synthetic construct
GRTFSNYAMG

SEQ ID NO: 80 - protein, 10 aa, synthetic construct
TISWNGGSTY

SEQ ID NO: 81 - protein, 19 aa, synthetic construct
RWLPVNQFLGVMRPSFVSA

SEQ ID NO: 82 - protein, 128 aa, synthetic construct
QLQLVESGGGLVQAGGSLRLSCAASGRTFSNYAMGWFRQAPGKEREFVATISWNGGSTYYEDSVKGRFTISRDNSENTVDLQMNSLKPEDTAVYYCAARWLPVNQFLGVMRPSFVSAWGQGTQVTVSS

SEQ ID NO: 83 - protein, 10 aa, synthetic construct
TRTFSHLAMG

SEQ ID NO: 84 - protein, 10 aa, synthetic construct
TISWGGDRTY

SEQ ID NO: 85 - protein, 17 aa, synthetic construct
DKLLFGWGSPPNTDFGS

SEQ ID NO: 86 - protein, 126 aa, synthetic construct
QVQLVESGGGLVQAGGSLRLSCAASTRTFSHLAMGWFRQAVGKEREPVATISWGGDRTYYADSVKARFAISRDNAKSTVYLQMNSLKPEDTAIYYCAADKLLFGWGSPPNTDFGSWGQGTQVTVSS

SEQ ID NO: 87 - protein, 11 aa, synthetic construct
GRRIFPLLTMG

SEQ ID NO: 88 - protein, 10 aa, synthetic construct
VIPRTGDSTY

SEQ ID NO: 89 - protein, 14 aa, synthetic construct
RDGSSSPRPADFGF

SEQ ID NO: 90 - protein, 124 aa, synthetic construct
QVQLVESGGGLVQAGDSLRLSCAVSGRRIFPLLTMGWFRQNPGKDREFVAVIPRTGDSTYYADSVKGRFAISRDNAKNTVHLQMNSLKPEDTAVYYCAARDGSSSPRPADFGFWGQGTQVTVSS

SEQ ID NO: 91 - protein, 10 aa, synthetic construct
GFTFSNHWMY

SEQ ID NO: 92 - protein, 10 aa, synthetic construct
DISPGGISTR

SEQ ID NO: 93 - protein, 16 aa, synthetic construct
GRAYVAGVSRASQYVY

SEQ ID NO: 94 - protein, 125 aa, synthetic construct
QLQLVESGGDLVQPGGSLRLSCLASGFTFSNHWMYWLRQAPGKGLEWVSDISPGGISTRYADSVKGRFTISRDNAKNTVYLEMSSLKPLDTAVYYCAAGRAYVAGVSRASQYVYWGQGTQVTVSS

SEQ ID NO: 95 - protein, 10 aa, synthetic construct
GRTFSHYTVG

SEQ ID NO: 96 - protein, 9 aa, synthetic construct
GLSWNHRTK

SEQ ID NO: 97 - protein, 15 aa, synthetic construct
DVSPFITTIQTDMEY

SEQ ID NO: 98 - protein, 123 aa, synthetic construct
QLQLVESGGGLVQPGGSLRLSCAASGRTFSHYTVGWFRQAPGKEREFVAGLSWNHRTKYADSVKGRFTISVDNAKNTVYLQMNSLKPEDTAVYVCTADVSPFITTIQTDMEYWGKGTLVTVSS

SEQ ID NO: 99 - protein, 10 aa, synthetic construct
GIIFSKHGMG

SEQ ID NO: 100 - protein, 9 aa, synthetic construct
RITSGGSTS

SEQ ID NO: 101 - protein, 15 aa, synthetic construct
ERFIINVEGAGRGPY

SEQ ID NO: 102 - protein, 123 aa, synthetic construct
QLQLVESGGGLVQSGGSLRLSCTTSGIIFSKHGMGWYRQAPGAQRELVARITSGGSTSYADSGKGRFTISRDNTKNTLYLQMNSLEPEDTAVYYCNVERFIINVEGAGRGPYWGQGTLVTVSS

SEQ ID NO: 103 - protein, 10 aa, synthetic construct
GRTFSTLNMG

SEQ ID NO: 104 - protein, 10 aa, synthetic construct
NIGWSGGTTY

SEQ ID NO: 105 - protein, 16 aa, synthetic construct
DIKGLYFPRDARSFDY

SEQ ID NO: 106 - protein, 125 aa, synthetic construct
QVQLVESGGGLVQAGGSLRLSCAVSGRTFSTLNMGWFRQAPGKEREFVANIGWSGGTTYSSDSAKGRFTISRDNAENTVYLQMNSLKPEDTAVYYCAADIKGLYFPRDARSFDYWGQGTQVTVSS

SEQ ID NO: 107 - protein, 10 aa, synthetic construct
GRIFPIYHMG

SEQ ID NO: 108 - protein, 10 aa, synthetic construct
AIRRSDSMTN

SEQ ID NO: 109 - protein, 14 aa, synthetic construct
ALGQYYGANTQYDS

SEQ ID NO: 110 - protein, 123 aa, synthetic construct
QLQLVESGGGLVQAGGSLRLSCAASGRIFPIYHMGWFRQAPGKEREFVAAIRRSDSMTNYADSVKGRFTISRDNAKNTLFLQMNSLRPEDTGVYNCAAALGQYYGANTQYDSWGQGTQVTVSS

SEQ ID NO: 111 - protein, 10 aa, synthetic construct
GSIFRFNLMG

SEQ ID NO: 112 - protein, 9 aa, synthetic construct
VMSEGGTTN

SEQ ID NO: 113 - protein, 11 aa, synthetic construct
WGSNSGPVLQY

SEQ ID NO: 114 - protein, 119 aa, synthetic construct
QLQLVESGGGLVQPGGSLRLSCAASGSIFRFNLMGWYRQAPGKQRELVAVMSEGGTTNYGDSVKGRFTMSRDNAKNTVYLQMNSLKSEDTAVYYCNFWGSNSGPVLQYWGQGTQVTVSS

SEQ ID NO: 115 - protein, 10 aa, synthetic construct
GRIFVISNAG

SEQ ID NO: 116 - protein, 10 aa, synthetic construct
SISRHGEITN

SEQ ID NO: 117 - protein, 15 aa, synthetic construct
TLGHSPRTDPGDFDS

SEQ ID NO: 118 - protein, 124 aa, synthetic construct
QVQLVESGGGSVQPGGSLRLACAASGRIFVISNAGWFRQTPGKEREFVASISRHGEITNYADAVKGRFTISRDNSKNMMYLQMNSLNFEDTAVYYCATTLGHSPRTDPGDFDSWGQGTQVTVSS

SEQ ID NO: 119 - protein, 10 aa, synthetic construct
GSIFRINTMG

SEQ ID NO: 120 - protein, 9 aa, synthetic construct
SFTSGGSPN

SEQ ID NO: 121 - protein, 15 aa, synthetic construct
YIMAWSHGVLKGYDS

SEQ ID NO: 122 - protein, 123 aa, synthetic construct
QVQLVESGGGLVQPGGSLRLSCAASGSIFRINTMGWYRQAPGKQRELVASFTSGGSPNYADSVKGRFTISRDNAKNTVYLQMNSLRPEETAVYYCNAYIMAWSHGVLKGYDSWGQGTQVTVSS

SEQ ID NO: 123 - protein, 10 aa, synthetic construct
GSIRTVNYMG

SEQ ID NO: 124 - protein, 9 aa, synthetic construct
VVTSGGGTN

SEQ ID NO: 125 - protein, 13 aa, synthetic construct
AASTYSSTVVRSF

SEQ ID NO: 126 - protein, 121 aa, synthetic construct
QVQLVESGGGLVQPGESLRLSCAASGSIRTVNYMGWHRQAPGKQRELVAVVTSGGGTNYADSVKGRFTISRDDTKNTVYLAMNSLKPEDTAVYYCNAAASTYSSTVVRSFWGQGTQVTVSS

SEQ ID NO: 127 - protein, 10 aa, synthetic construct
GSIFRINSMG

SEQ ID NO: 128 - protein, 10 aa, synthetic construct
TFTTSGGVTN

SEQ ID NO: 129 - protein, 15 aa, synthetic construct
YVMAWSRGVLKGYDS

SEQ ID NO: 130 - protein, 124 aa, synthetic construct
QVQLVESGGGLVQPGGSLRLSCAASGSIFRINSMGWYRQAPGKQRELVATFTTSGGVTNYADSVKGRFTISRDNAKNTVYLQMNNLTPEETAVYYCNAYVMAWSRGVLKGYDSWGQGTQVTVSS

SEQ ID NO: 131 - protein, 10 aa, synthetic construct
GRTFSGYRMG

SEQ ID NO: 132 - protein, 10 aa, synthetic construct
SIRWIGPATA

SEQ ID NO: 133 - protein, 14 aa, synthetic construct
DPTPSIDYKRGYDY

SEQ ID NO: 134 - protein, 123 aa, synthetic construct
QVQLVESGGGLVQAGGSLRLSCAASGRTFSGYRMGWFRQAPGKEREFVASIRWIGPATAYADSVKGRFTISRDNAKNTVYLQMNSLKSEDTAVYYCAADPTPSIDYKRGYDYWGQGTQVTVSS

SEQ ID NO: 135 - protein, 10 aa, synthetic construct
GRTFNTFRTG

SEQ ID NO: 136 - protein, 10 aa, synthetic construct
SLNWSSTWTS

SEQ ID NO: 137 - protein, 15 aa, synthetic construct
GIAGTPVMRATSYIY

SEQ ID NO: 138 - protein, 124 aa, synthetic construct
QVQLVESGGGLVQPGGSLRVSCAASGRTFNTFRTGWFRQAPGKEREFVASLNWSSTWTSYADSVKGRFSISRDSAKNTVYLQMNSLKPEDTADYYCAVGIAGTPVMRATSYIYWGQGTQVTVSS

SEQ ID NO: 139 - protein, 10 aa, synthetic construct
RFIFPIYAMG

SEQ ID NO: 140 - protein, 10 aa, synthetic construct
GIERTTDTTL

SEQ ID NO: 141 - protein, 14 aa, synthetic construct
RNSRRIGDVNDVDY

SEQ ID NO: 142 - protein, 123 aa, synthetic construct
QVQLVESGGGLVQPGGSLRLSCAASRFIFPIYAMGWFRQAPGKEREFVAGIERTTDTTLYADSVKGRFTISRDNAKNTVYLQMYSLKPEDAAVYYCAARNSRRIGDVNDVDYWGQGTQVTVSS

SEQ ID NO: 143 - protein, 10 aa, synthetic construct
RTIFPLYAMG

SEQ ID NO: 144 - protein, 10 aa, synthetic construct
GISRTTSTTL

SEQ ID NO: 145 - protein, 14 aa, synthetic construct
RNSRTIGDVNDVDY

SEQ ID NO: 146 - protein, 123 aa, synthetic construct
QLQLVESGGGLVQAGGSLRLSCAASRTIFPLYAMGWFRQAPGKEREFVAGISRTTSTTLYADSVKGRFTISRDNAANTVYLQMNTLKPEDAAVYYCAARNSRTIGDVNDVDYWGQGTQLTVSS

SEQ ID NO: 147 - protein, 10 aa, synthetic construct
GRTISIYMMG

SEQ ID NO: 148 - protein, 10 aa, synthetic construct
AIMPSGSRTY

SEQ ID NO: 149 - protein, 15 aa, synthetic construct
KLFRGSGDYINDYDH

SEQ ID NO: 150 - protein, 124 aa, synthetic construct
QVQLVESGGGLVQAGGSLRLSCAASGRTISIYMMGWFRQAPGKGREFVSAIMPSGSRTYSADWVKGRFTISRDNSKSTVYLQMNSLKPEDTAVYYCAAKLFRGSGDYINDYDHWGQGTQVTVSS

SEQ ID NO: 151 - protein, 121 aa, synthetic construct
QVQLVESGGGLVQPGGSLRLSCAASGSIRTVNYMGWHRQAPGKQRELVAVVTSGGGTNYADSVKGRFTISRDDTKNTVYLQMNSLRAEDTAVYYCNAAASTYSSTVVRSFWGQGTLVTVSS

SEQ ID NO: 152 - protein, 121 aa, synthetic construct
QVQLVESGGGLVQPGGSLRLSCAASGSIRTVNYMGWHRQAPGKQRELVAVVTSGGGTNYADSVKGRFTISRDNTKNTVYLQMNSLRAEDTAVYYCNAAASTYSSTVVRSFWGQGTLVTVSS

SEQ ID NO: 153 - protein, 121 aa, synthetic construct
QVQLVESGGGLVQPGGSLRLSCAASGSIRTVNYMGWHRQAPGKQRELVAVVTSGGGTNYADSVKGRFTISRDDSKNTVYLQMNSLRAEDTAVYYCNAAASTYSSTVVRSFWGQGTLVTVSS

SEQ ID NO: 154 - protein, 121 aa, synthetic construct
QVQLVESGGGLVQPGGSLRLSCAASGSIRTVNYMGWHRQAPGKQRELVAVVTSGGGTNYADSVKGRFTISRDNSKNTVYLQMNSLRAEDTAVYYCNAAASTYSSTVVRSFWGQGTLVTVSS

SEQ ID NO: 155 - protein, 121 aa, synthetic construct
QVQLVESGGGLVQPGGSLRLSCAASGSIRTVNYMGWHRQAPGKGRELVAVVTSGGGTNYADSVKGRFTISRDDTKNTVYLQMNSLRAEDTAVYYCNAAASTYSSTVVRSFWGQGTLVTVSS

SEQ ID NO: 156 - protein, 121 aa, synthetic construct
QVQLVESGGGLVQPGGSLRLSCAASGSIRTVNYMGWHRQAPGKQLELVAVVTSGGGTNYADSVKGRFTISRDDTKNTVYLQMNSLRAEDTAVYYCNAAASTYSSTVVRSFWGQGTLVTVSS

SEQ ID NO: 157 - protein, 121 aa, synthetic construct
EVQLVESGGGLVQPGGSLRLSCAASGSIRTVNYMGWHRQAPGKQRELVAVVTSGGGTNYADSVKGRFTISRDDTKNTVYLQMNSLRAEDTAVYYCNAAASTYSSTVVRSFWGQGTLVTVSS

SEQ ID NO: 158 - protein, 121 aa, synthetic construct
QVQLVESGGGLVQPGGSLRLSCAASGSIRTVNYMGWHRQAPGKQRELVSVVTSGGGTNYADSVKGRFTISRDDTKNTVYLQMNSLRAEDTAVYYCNAAASTYSSTVVRSFWGQGTLVTVSS

SEQ ID NO: 159 - protein, 232 aa, synthetic construct
EPKSCDKTHTCPPCPAPELLGGPSVFLFPPKPKDTLMISRTPEVTCVVVDVSHEDPEVKFNWYVDGVEVHNAKTKPREEQYNSTYRVVSVLTVLHQDWLNGKEYKCKVSNKALPAPIEKTISKAKGQPREPQVYTLPPSREEMTKNQVSLTCLVKGFYPSDIAVEWESNGQPENNYKTTPPVLDSDGSFFLYSKLTVDKSRWQQGNVFSCSVMHEALHNHYTQKSLSLSPGK

SEQ ID NO: 160 - protein, 232 aa, synthetic construct
EPKSADKTHTCPPCPAPEAAGGPSVFLFPPKPKDTLMISRTPEVTCVVVDVSHEDPEVKFNWYVDGVEVHNAKTKPREEQYNSTYRVVSVLTVLHQDWLNGKEYKCKVSNKALPAPIEKTISKAKGQPREPQVYTLPPSREEMTKNQVSLTCLVKGFYPSDIAVEWESNGQPENNYKTTPPVLDSDGSFFLYSKLTVDKSRWQQGNVFSCSVMHEALHNHYTQKSLSLSPGK

SEQ ID NO: 161 - protein, 347 aa, synthetic construct
QVQLVESGGGLVQPGGSLTLSCVAAGSNFSLYAMSYYRQVPGKQRELVARIRDNGRTNYADSVKDRFTISRDSAKNTVYLQMHSLKPEDTAVYYCNADNRVTTFWGRGTQVTVSSEPKSADKTHTCPPCPAPEAAGGPSVFLFPPKPKDTLMISRTPEVTCVVVDVSHEDPEVKFNWYVDGVEVHNAKTKPREEQYNSTYRVVSVLTVLHQDWLNGKEYKCKVSNKALPAPIEKTISKAKGQPREPQVYTLPPSREEMTKNQVSLTCLVKGFYPSDIAVEWESNGQPENNYKTTPPVLDSDGSFFLYSKLTVDKSRWQQGNVFSCSVMHEALHNHYTQKSLSLSPGK

SEQ ID NO: 162 - protein, 347 aa, synthetic construct
QLQLVESGGGLVQPGGSLRLSCAASGSIFSIDAMGWYRQAPGKERELVAAIGSGTYYADSVKGRFTISRDNAKKNTLYLQMDSLKPEDTAIYYCASGDSYPDEYWGQGTQVTVSAEPKSADKTHTCPPCPAPEAAGGPSVFLFPPKPKDTLMISRTPEVTCVVVDVSHEDPEVKFNWYVDGVEVHNAKTKPREEQYNSTYRVVSVLTVLHQDWLNGKEYKCKVSNKALPAPIEKTISKAKGQPREPQVYTLPPSREEMTKNQVSLTCLVKGFYPSDIAVEWESNGQPENNYKTTPPVLDSDGSFFLYSKLTVDKSRWQQGNVFSCSVMHEALHNHYTQKSLSLSPGK

SEQ ID NO: 163 - protein, 349 aa, synthetic construct
QLQLVESGGGLVQPGGSLRLSCAASESDFSIYIMGWYRQAPGKQRELVVTITPGGNTNYVDSVKGRFTISRDNTMNTAYLQMNSLKPDDTAVYYCNARNIFRNVDYSGKGTLVTVSSEPKSADKTHTCPPCPAPEAAGGPSVFLFPPKPKDTLMISRTPEVTCVVVDVSHEDPEVKFNWYVDGVEVHNAKTKPREEQYNSTYRVVSVLTVLHQDWLNGKEYKCKVSNKALPAPIEKTISKAKGQPREPQVYTLPPSREEMTKNQVSLTCLVKGFYPSDIAVEWESNGQPENNYKTTPPVLDSDGSFFLYSKLTVDKSRWQQGNVFSCSVMHEALHNHYTQKSLSLSPGK

SEQ ID NO: 164 - protein, 349 aa, synthetic construct
QVQLVESGGGLVQPGGSLRLSCVASGIEFSIYIMGWYRQAPGKQRELVATVTPGGNTNYADSVKGRFTISRDNTKNTAYLQMNSLKPDDTAVYYCNARNIFRNMDYQGKGTLVTVSSEPKSADKTHTCPPCPAPEAAGGPSVFLFPPKPKDTLMISRTPEVTCVVVDVSHEDPEVKFNWYVDGVEVHNAKTKPREEQYNSTYRVVSVLTVLHQDWLNGKEYKCKVSNKALPAPIEKTISKAKGQPREPQVYTLPPSREEMTKNQVSLTCLVKGFYPSDIAVEWESNGQPENNYKTTPPVLDSDGSFFLYSKLTVDKSRWQQGNVFSCSVMHEALHNHYTQKSLSLSPGK

SEQ ID NO: 165 - protein, 349 aa, synthetic construct
QVQLVESGGGSVQPGGSLRLSCAASGSDFNIYIMGWYQQAPGKQRELVATITPGGNTNYVDSVKGRFTISRDNTKNTAYLQMNSLKPDDTAVYYCNARNIFRYMDYWGKGTLVTVSSEPKSADKTHTCPPCPAPEAAGGPSVFLFPPKPKDTLMISRTPEVTCVVVDVSHEDPEVKFNWYVDGVEVHNAKTKPREEQYNSTYRVVSVLTVLHQDWLNGKEYKCKVSNKALPAPIEKTISKAKGQPREPQVYTLPPSREEMTKNQVSLTCLVKGFYPSDIAVEWESNGQPENNYKTTPPVLDSDGSFFLYSKLTVDKSRWQQGNVFSCSVMHEALHNHYTQKSLSLSPGK

SEQ ID NO: 166 - protein, 364 aa, synthetic construct
QVQLVESGGGLVQAGGSLRLSCAASGFIFDDYAIAWFRQAPGKEREGVSFISNSDGTAYYADSVKGRFTISSDNAKNTVYLQMDSLKPDDTADYYCAAEGRMGTHSRDSVYFWAFSALYDYWGQGTQVTVSSEPKSADKTHTCPPCPAPEAAGGPSVFLFPPKPKDTLMISRTPEVTCVVVDVSHEDPEVKFNWYVDGVEVHNAKTKPREEQYNSTYRVVSVLTVLHQDWLNGKEYKCKVSNKALPAPIEKTISKAKGQPREPQVYTLPPSREEMTKNQVSLTCLVKGFYPSDIAVEWESNGQPENNYKTTPPVLDSDGSFFLYSKLTVDKSRWQQGNVFSCSVMHEALHNHYTQKSLSLSPGK

SEQ ID NO: 167 - protein, 364 aa, synthetic construct
QLQLVESGGGLVQAGGSLRLSCAASGFTFDDYAITWFRQAPGKEREGVAYISNSDGMTYYVDSVKGRFTISSDNAKNTVYLQMDSLKPEDTAVYYCAAEGIMGTHNRDNVYFWAFSALYDYWGQGTQVTVSSEPKSADKTHTCPPCPAPEAAGGPSVFLFPPKPKDTLMISRTPEVTCVVVDVSHEDPEVKFNWYVDGVEVHNAKTKPREEQYNSTYRVVSVLTVLHQDWLNGKEYKCKVSNKALPAPIEKTISKAKGQPREPQVYTLPPSREEMTKNQVSLTCLVKGFYPSDIAVEWESNGQPENNYKTTPPVLDSDGSFFLYSKLTVDKSRWQQGNVFSCSVMHEALHNHYTQKSLSLSPGK

SEQ ID NO: 168 - protein, 364 aa, synthetic construct
QVQLVESGGGLVQAGGSLRLSCAASGFTFDDYAITWFRQAPGKEREGVAYISNFDGMTYYADSVKGRFTISSDNAKNTVYLQMDSLKPEDTAVYYCAAEGRMGTHSRDSVYFWAFSALYDHWGQGTQVTVSSEPKSADKTHTCPPCPAPEAAGGPSVFLFPPKPKDTLMISRTPEVTCVVVDVSHEDPEVKFNWYVDGVEVHNAKTKPREEQYNSTYRVVSVLTVLHQDWLNGKEYKCKVSNKALPAPIEKTISKAKGQPREPQVYTLPPSREEMTKNQVSLTCLVKGFYPSDIAVEWESNGQPENNYKTTPPVLDSDGSFFLYSKLTVDKSRWQQGNVFSCSVMHEALHNHYTQKSLSLSPGK

SEQ ID NO: 169 - protein, 364 aa, synthetic construct
QVQLVESGGGLVQAGGSLRLSCAASGFTFDDYAITWFRQAPGKEREGVAYISNSDGMTYYADSVKGRFTISSDNAKNTVYLQMDSLKPEDTAVYYCAAEGRMGTHSRDSVYFWAFSALYDYWGQGTQVTVSSEPKSADKTHTCPPCPAPEAAGGPSVFLFPPKPKDTLMISRTPEVTCVVVDVSHEDPEVKFNWYVDGVEVHNAKTKPREEQYNSTYRVVSVLTVLHQDWLNGKEYKCKVSNKALPAPIEKTISKAKGQPREPQVYTLPPSREEMTKNQVSLTCLVKGFYPSDIAVEWESNGQPENNYKTTPPVLDSDGSFFLYSKLTVDKSRWQQGNVFSCSVMHEALHNHYTQKSLSLSPGK

SEQ ID NO: 170 - protein, 364 aa, synthetic construct
QVQLVESGGGLVQAGGSLRLSCAASGFTFDDYAITWFRQAPGKEREGVAYISNNDGMTYYADSVKGRFTISSDNAKNPVYLQMDSLKPEDTAVYYCAAEGRMGTHSRDSVYFWAFSALYDYWGQGTQVTVSSEPKSADKTHTCPPCPAPEAAGGPSVFLFPPKPKDTLMISRTPEVTCVVVDVSHEDPEVKFNWYVDGVEVHNAKTKPREEQYNSTYRVVSVLTVLHQDWLNGKEYKCKVSNKALPAPIEKTISKAKGQPREPQVYTLPPSREEMTKNQVSLTCLVKGFYPSDIAVEWESNGQPENNYKTTPPVLDSDGSFFLYSKLTVDKSRWQQGNVFSCSVMHEALHNHYTQKSLSLSPGK

SEQ ID NO: 171 - protein, 364 aa, synthetic construct
QVQLVESGGGLVQAGGSLRLSCAASGFTFGDYAITWFRQAPGKEREGVAYISNFDGMTYYADSVKGRFTISSDNAKNTVYLQMDSLKPEDTAVYYCAAEGRMGTHSRDSVYFWAFSALYDYWGQGTQVTVSSEPKSADKTHTCPPCPAPEAAGGPSVFLFPPKPKDTLMISRTPEVTCVVVDVSHEDPEVKFNWYVDGVEVHNAKTKPREEQYNSTYRVVSVLTVLHQDWLNGKEYKCKVSNKALPAPIEKTISKAKGQPREPQVYTLPPSREEMTKNQVSLTCLVKGFYPSDIAVEWESNGQPENNYKTTPPVLDSDGSFFLYSKLTVDKSRWQQGNVFSCSVMHEALHNHYTQKSLSLSPGK

SEQ ID NO: 172 - protein, 364 aa, synthetic construct
QVQLVESGGGLVQAGGSLRLSCAASGFIFDDYAIAWFRQAPGKEREGVSFISNSDGTAYYADSVKGRFTISSDNAKNTVYLQMDSLKPDDTADYYCAAEGRMGTHSGDSVYFWSFSALYDYWGQGTQVTVSSEPKSADKTHTCPPCPAPEAAGGPSVFLFPPKPKDTLMISRTPEVTCVVVDVSHEDPEVKFNWYVDGVEVHNAKTKPREEQYNSTYRVVSVLTVLHQDWLNGKEYKCKVSNKALPAPIEKTISKAKGQPREPQVYTLPPSREEMTKNQVSLTCLVKGFYPSDIAVEWESNGQPENNYKTTPPVLDSDGSFFLYSKLTVDKSRWQQGNVFSCSVMHEALHNHYTQKSLSLSPGK

SEQ ID NO: 173 - protein, 364 aa, synthetic construct
QLQLVESGGGLVQAGGSLRLSCAASGFNFDDYAIAWFRQAPGKEREGVSFISNSDGTAYYADSVKGRFTISSDNAKNTVYLQMDSLKPDDTADYYCAAEGRMGTHSRDSVYFWSFSALYDYWGQGTQVTVSSEPKSADKTHTCPPCPAPEAAGGPSVFLFPPKPKDTLMISRTPEVTCVVVDVSHEDPEVKFNWYVDGVEVHNAKTKPREEQYNSTYRVVSVLTVLHQDWLNGKEYKCKVSNKALPAPIEKTISKAKGQPREPQVYTLPPSREEMTKNQVSLTCLVKGFYPSDIAVEWESNGQPENNYKTTPPVLDSDGSFFLYSKLTVDKSRWQQGNVFSCSVMHEALHNHYTQKSLSLSPGK

SEQ ID NO: 174 - protein, 364 aa, synthetic construct
QVQLVESGGGLVQAGGSLRLSCAASGFSFDDYAIAWFRQAPGKEREGVSFISNSDGTAYYADSVKGRFTISSDNAKNTVYLQMDSLKPDDTADYYCAAEGRMGTHSRDSVYFWSFSALYDYWGQGTQVTVSSEPKSADKTHTCPPCPAPEAAGGPSVFLFPPKPKDTLMISRTPEVTCVVVDVSHEDPEVKFNWYVDGVEVHNAKTKPREEQYNSTYRVVSVLTVLHQDWLNGKEYKCKVSNKALPAPIEKTISKAKGQPREPQVYTLPPSREEMTKNQVSLTCLVKGFYPSDIAVEWESNGQPENNYKTTPPVLDSDGSFFLYSKLTVDKSRWQQGNVFSCSVMHEALHNHYTQKSLSLSPGK

SEQ ID NO: 175 - protein, 364 aa, synthetic construct
QLQLVESGGGLVQPGGSLRLSCVLSGGTFERLAMGWFRQAPGKEREGVSFISNSDGTAYYADSVKGRFTISSDNAKNTVYLQMDSLKPDDTADYYCAAEGRMGTHSRDSVYFWSFSALYDYWGQGTQVTVSAEPKSADKTHTCPPCPAPEAAGGPSVFLFPPKPKDTLMISRTPEVTCVVVDVSHEDPEVKFNWYVDGVEVHNAKTKPREEQYNSTYRVVSVLTVLHQDWLNGKEYKCKVSNKALPAPIEKTISKAKGQPREPQVYTLPPSREEMTKNQVSLTCLVKGFYPSDIAVEWESNGQPENNYKTTPPVLDSDGSFFLYSKLTVDKSRWQQGNVFSCSVMHEALHNHYTQKSLSLSPGK

SEQ ID NO: 176 - protein, 364 aa, synthetic construct
QVQLVESGGGLVQAGGSLRLSCAASGFTFDDYAITWFRQAPGKEREGVSYISNNDHNTYYADSVKGRFTISSDNAKNTVYLQMDSLKPEDTAVYYCAAEGRMGTHSRESSYFWTFPALYDYWGQGTQVTVSSEPKSADKTHTCPPCPAPEAAGGPSVFLFPPKPKDTLMISRTPEVTCVVVDVSHEDPEVKFNWYVDGVEVHNAKTKPREEQYNSTYRVVSVLTVLHQDWLNGKEYKCKVSNKALPAPIEKTISKAKGQPREPQVYTLPPSREEMTKNQVSLTCLVKGFYPSDIAVEWESNGQPENNYKTTPPVLDSDGSFFLYSKLTVDKSRWQQGNVFSCSVMHEALHNHYTQKSLSLSPGK

SEQ ID NO: 177 - protein, 364 aa, synthetic construct
QVQLLESGGGLVQPGGSLRLSCAASGFTFGDYAITWFRQAPGKGLEGVAYISNFDGMTYYADSVKGRFTISSDNSKNTVYLQMNSLRAEDTAVYYCAAEGRMGTHSRDSVYFWAFSALYDYWGQGTLVTVSSEPKSADKTHTCPPCPAPEAAGGPSVFLFPPKPKDTLMISRTPEVTCVVVDVSHEDPEVKFNWYVDGVEVHNAKTKPREEQYNSTYRVVSVLTVLHQDWLNGKEYKCKVSNKALPAPIEKTISKAKGQPREPQVYTLPPSREEMTKNQVSLTCLVKGFYPSDIAVEWESNGQPENNYKTTPPVLDSDGSFFLYSKLTVDKSRWQQGNVFSCSVMHEALHNHYTQKSLSLSPGK

SEQ ID NO: 178 - protein, 364 aa, synthetic construct
EVQLLESGGGLVQPGGSLRLSCAASGFTFGDYAITWFRQAPGKGLEGVAYISNFDGMTYYADSVKGRFTISSDNSKNTVYLQMNSLRAEDTAVYYCAAEGRMGTHSRDSVYFWAFSALYDYWGQGTLVTVSSEPKSADKTHTCPPCPAPEAAGGPSVFLFPPKPKDTLMISRTPEVTCVVVDVSHEDPEVKFNWYVDGVEVHNAKTKPREEQYNSTYRVVSVLTVLHQDWLNGKEYKCKVSNKALPAPIEKTISKAKGQPREPQVYTLPPSREEMTKNQVSLTCLVKGFYPSDIAVEWESNGQPENNYKTTPPVLDSDGSFFLYSKLTVDKSRWQQGNVFSCSVMHEALHNHYTQKSLSLSPGK

SEQ ID NO: 179 - protein, 364 aa, synthetic construct
QVQLLESGGGLVQPGGSLRLSCAASGFTFGDYAITWFRQAPGKGLEGVAYISNFDGMTYYADSVKGRFTISRDNSKNTVYLQMNSLRAEDTAVYYCAAEGRMGTHSRDSVYFWAFSALYDYWGQGTLVTVSSEPKSADKTHTCPPCPAPEAAGGPSVFLFPPKPKDTLMISRTPEVTCVVVDVSHEDPEVKFNWYVDGVEVHNAKTKPREEQYNSTYRVVSVLTVLHQDWLNGKEYKCKVSNKALPAPIEKTISKAKGQPREPQVYTLPPSREEMTKNQVSLTCLVKGFYPSDIAVEWESNGQPENNYKTTPPVLDSDGSFFLYSKLTVDKSRWQQGNVFSCSVMHEALHNHYTQKSLSLSPGK

SEQ ID NO: 180 - protein, 364 aa, synthetic construct
EVQLLESGGGLVQPGGSLRLSCAASGFTFGDYAITWFRQAPGKGLEGVAYISNFDGMTYYADSVKGRFTISRDNSKNTVYLQMNSLRAEDTAVYYCAAEGRMGTHSRDSVYFWAFSALYDYWGQGTLVTVSSEPKSADKTHTCPPCPAPEAAGGPSVFLFPPKPKDTLMISRTPEVTCVVVDVSHEDPEVKFNWYVDGVEVHNAKTKPREEQYNSTYRVVSVLTVLHQDWLNGKEYKCKVSNKALPAPIEKTISKAKGQPREPQVYTLPPSREEMTKNQVSLTCLVKGFYPSDIAVEWESNGQPENNYKTTPPVLDSDGSFFLYSKLTVDKSRWQQGNVFSCSVMHEALHNHYTQKSLSLSPGK

SEQ ID NO: 181 - protein, 364 aa, synthetic construct
EVQLLESGGGLVQAGGSLRLSCAASGFTFGDYAITWFRQAPGKGLEGVAYISNFDGMTYYADSVKGRFTISSDNSKNTVYLQMNSLRAEDTAVYYCAAEGRMGTHSRDSVYFWAFSALYDYWGQGTLVTVSSEPKSADKTHTCPPCPAPEAAGGPSVFLFPPKPKDTLMISRTPEVTCVVVDVSHEDPEVKFNWYVDGVEVHNAKTKPREEQYNSTYRVVSVLTVLHQDWLNGKEYKCKVSNKALPAPIEKTISKAKGQPREPQVYTLPPSREEMTKNQVSLTCLVKGFYPSDIAVEWESNGQPENNYKTTPPVLDSDGSFFLYSKLTVDKSRWQQGNVFSCSVMHEALHNHYTQKSLSLSPGK

SEQ ID NO: 182 - protein, 364 aa, synthetic construct
EVQLLESGGGLVQPGGSLRLSCAASGFTFGDYAITWFRQAPGKELEGVAYISNFDGMTYYADSVKGRFTISSDNSKNTVYLQMNSLRAEDTAVYYCAAEGRMGTHSRDSVYFWAFSALYDYWGQGTLVTVSSEPKSADKTHTCPPCPAPEAAGGPSVFLFPPKPKDTLMISRTPEVTCVVVDVSHEDPEVKFNWYVDGVEVHNAKTKPREEQYNSTYRVVSVLTVLHQDWLNGKEYKCKVSNKALPAPIEKTISKAKGQPREPQVYTLPPSREEMTKNQVSLTCLVKGFYPSDIAVEWESNGQPENNYKTTPPVLDSDGSFFLYSKLTVDKSRWQQGNVFSCSVMHEALHNHYTQKSLSLSPGK

SEQ ID NO: 183 - protein, 364 aa, synthetic construct
EVQLLESGGGLVQPGGSLRLSCAASGFTFGDYAITWFRQAPGKGREGVAYISNFDGMTYYADSVKGRFTISSDNSKNTVYLQMNSLRAEDTAVYYCAAEGRMGTHSRDSVYFWAFSALYDYWGQGTLVTVSSEPKSADKTHTCPPCPAPEAAGGPSVFLFPPKPKDTLMISRTPEVTCVVVDVSHEDPEVKFNWYVDGVEVHNAKTKPREEQYNSTYRVVSVLTVLHQDWLNGKEYKCKVSNKALPAPIEKTISKAKGQPREPQVYTLPPSREEMTKNQVSLTCLVKGFYPSDIAVEWESNGQPENNYKTTPPVLDSDGSFFLYSKLTVDKSRWQQGNVFSCSVMHEALHNHYTQKSLSLSPGK

SEQ ID NO: 184 - protein, 364 aa, synthetic construct
EVQLLESGGGLVQPGGSLRLSCAASGFTFGDYAITWFRQAPGKEREGVAYISNFDGMTYYADSVKGRFTISSDNSKNTVYLQMNSLRAEDTAVYYCAAEGRMGTHSRDSVYFWAFSALYDYWGQGTLVTVSSEPKSADKTHTCPPCPAPEAAGGPSVFLFPPKPKDTLMISRTPEVTCVVVDVSHEDPEVKFNWYVDGVEVHNAKTKPREEQYNSTYRVVSVLTVLHQDWLNGKEYKCKVSNKALPAPIEKTISKAKGQPREPQVYTLPPSREEMTKNQVSLTCLVKGFYPSDIAVEWESNGQPENNYKTTPPVLDSDGSFFLYSKLTVDKSRWQQGNVFSCSVMHEALHNHYTQKSLSLSPGK

SEQ ID NO: 185 - protein, 364 aa, synthetic construct
EVQLLESGGGLVQPGGSLRLSCAASGFTFGDYAITWFRQAPGKGLEGVAYISNFDGMTYYADSVKGRFTISSDNAKNTVYLQMNSLRAEDTAVYYCAAEGRMGTHSRDSVYFWAFSALYDYWGQGTLVTVSSEPKSADKTHTCPPCPAPEAAGGPSVFLFPPKPKDTLMISRTPEVTCVVVDVSHEDPEVKFNWYVDGVEVHNAKTKPREEQYNSTYRVVSVLTVLHQDWLNGKEYKCKVSNKALPAPIEKTISKAKGQPREPQVYTLPPSREEMTKNQVSLTCLVKGFYPSDIAVEWESNGQPENNYKTTPPVLDSDGSFFLYSKLTVDKSRWQQGNVFSCSVMHEALHNHYTQKSLSLSPGK

SEQ ID NO: 186 - protein, 364 aa, synthetic construct
EVQLLESGGGLVQPGGSLRLSCAASGFTFGDYAITWFRQAPGKGLEGVAYISNFDGMTYYADSVKGRFTISSDNSKNTVYLQMDSLRAEDTAVYYCAAEGRMGTHSRDSVYFWAFSALYDYWGQGTLVTVSSEPKSADKTHTCPPCPAPEAAGGPSVFLFPPKPKDTLMISRTPEVTCVVVDVSHEDPEVKFNWYVDGVEVHNAKTKPREEQYNSTYRVVSVLTVLHQDWLNGKEYKCKVSNKALPAPIEKTISKAKGQPREPQVYTLPPSREEMTKNQVSLTCLVKGFYPSDIAVEWESNGQPENNYKTTPPVLDSDGSFFLYSKLTVDKSRWQQGNVFSCSVMHEALHNHYTQKSLSLSPGK

SEQ ID NO: 187 - protein, 364 aa, synthetic construct
EVQLLESGGGLVQPGGSLRLSCAASGFTFGDYAITWFRQAPGKGLEGVAYISNFDGMTYYADSVKGRFTISSDNSKNTVYLQMNSLRPEDTAVYYCAAEGRMGTHSRDSVYFWAFSALYDYWGQGTLVTVSSEPKSADKTHTCPPCPAPEAAGGPSVFLFPPKPKDTLMISRTPEVTCVVVDVSHEDPEVKFNWYVDGVEVHNAKTKPREEQYNSTYRVVSVLTVLHQDWLNGKEYKCKVSNKALPAPIEKTISKAKGQPREPQVYTLPPSREEMTKNQVSLTCLVKGFYPSDIAVEWESNGQPENNYKTTPPVLDSDGSFFLYSKLTVDKSRWQQGNVFSCSVMHEALHNHYTQKSLSLSPGK

SEQ ID NO: 188 - protein, 364 aa, synthetic construct
EVQLLESGGGLVQPGGSLRLSCAASGFTFGDYAITWFRQAPGKGLEGVSYISNFDGMTYYADSVKGRFTISSDNSKNTVYLQMNSLRAEDTAVYYCAAEGRMGTHSRDSVYFWAFSALYDYWGQGTLVTVSSEPKSADKTHTCPPCPAPEAAGGPSVFLFPPKPKDTLMISRTPEVTCVVVDVSHEDPEVKFNWYVDGVEVHNAKTKPREEQYNSTYRVVSVLTVLHQDWLNGKEYKCKVSNKALPAPIEKTISKAKGQPREPQVYTLPPSREEMTKNQVSLTCLVKGFYPSDIAVEWESNGQPENNYKTTPPVLDSDGSFFLYSKLTVDKSRWQQGNVFSCSVMHEALHNHYTQKSLSLSPGK

SEQ ID NO: 189 - protein, 364 aa, synthetic construct
EVQLVESGGGLVQPGGSLRLSCAASGFTFGDYAITWFRQAPGKGLEGVAYISNFDGMTYYADSVKGRFTISSDNSKNTVYLQMNSLRAEDTAVYYCAAEGRMGTHSRDSVYFWAFSALYDYWGQGTLVTVSSEPKSADKTHTCPPCPAPEAAGGPSVFLFPPKPKDTLMISRTPEVTCVVVDVSHEDPEVKFNWYVDGVEVHNAKTKPREEQYNSTYRVVSVLTVLHQDWLNGKEYKCKVSNKALPAPIEKTISKAKGQPREPQVYTLPPSREEMTKNQVSLTCLVKGFYPSDIAVEWESNGQPENNYKTTPPVLDSDGSFFLYSKLTVDKSRWQQGNVFSCSVMHEALHNHYTQKSLSLSPGK

SEQ ID NO: 190 - protein, 364 aa, synthetic construct
EVQLLESGGGLVQPGGSLRLSCAASGFTFGDYAITWVRQAPGKGLEGVAYISNFDGMTYYADSVKGRFTISSDNSKNTVYLQMNSLRAEDTAVYYCAAEGRMGTHSRDSVYFWAFSALYDYWGQGTLVTVSSEPKSADKTHTCPPCPAPEAAGGPSVFLFPPKPKDTLMISRTPEVTCVVVDVSHEDPEVKFNWYVDGVEVHNAKTKPREEQYNSTYRVVSVLTVLHQDWLNGKEYKCKVSNKALPAPIEKTISKAKGQPREPQVYTLPPSREEMTKNQVSLTCLVKGFYPSDIAVEWESNGQPENNYKTTPPVLDSDGSFFLYSKLTVDKSRWQQGNVFSCSVMHEALHNHYTQKSLSLSPGK

SEQ ID NO: 191 - protein, 360 aa, synthetic construct
QLQLVESGGGLVQAGGSLRLSCAASGRTFSNYAMGWFRQAPGKEREFVATISWNGGSTYYEDSVKGRFTISRDNSENTVDLQMNSLKPEDTAVYYCAARWLPVNQFLGVMRPSFVSAWGQGTQVTVSSEPKSADKTHTCPPCPAPEAAGGPSVFLFPPKPKDTLMISRTPEVTCVVVDVSHEDPEVKFNWYVDGVEVHNAKTKPREEQYNSTYRVVSVLTVLHQDWLNGKEYKCKVSNKALPAPIEKTISKAKGQPREPQVYTLPPSREEMTKNQVSLTCLVKGFYPSDIAVEWESNGQPENNYKTTPPVLDSDGSFFLYSKLTVDKSRWQQGNVFSCSVMHEALHNHYTQKSLSLSPGK

SEQ ID NO: 192 - protein, 358 aa, synthetic construct
QVQLVESGGGLVQAGGSLRLSCAASTRTFSHLAMGWFRQAVGKEREPVATISWGGDRTYYADSVKARFAISRDNAKSTVYLQMNSLKPEDTAIYYCAADKLLFGWGSPPNTDFGSWGQGTQVTVSSEPKSADKTHTCPPCPAPEAAGGPSVFLFPPKPKDTLMISRTPEVTCVVVDVSHEDPEVKFNWYVDGVEVHNAKTKPREEQYNSTYRVVSVLTVLHQDWLNGKEYKCKVSNKALPAPIEKTISKAKGQPREPQVYTLPPSREEMTKNQVSLTCLVKGFYPSDIAVEWESNGQPENNYKTTPPVLDSDGSFFLYSKLTVDKSRWQQGNVFSCSVMHEALHNHYTQKSLSLSPGK

SEQ ID NO: 193 - protein, 356 aa, synthetic construct
QVQLVESGGGLVQAGDSLRLSCAVSGRRIFPLLTMGWFRQNPGKDREFVAVIPRTGDSTYYADSVKGRFAISRDNAKNTVHLQMNSLKPEDTAVYYCAARDGSSSPRPADFGFWGQGTQVTVSSEPKSADKTHTCPPCPAPEAAGGPSVFLFPPKPKDTLMISRTPEVTCVVVDVSHEDPEVKFNWYVDGVEVHNAKTKPREEQYNSTYRVVSVLTVLHQDWLNGKEYKCKVSNKALPAPIEKTISKAKGQPREPQVYTLPPSREEMTKNQVSLTCLVKGFYPSDIAVEWESNGQPENNYKTTPPVLDSDGSFFLYSKLTVDKSRWQQGNVFSCSVMHEALHNHYTQKSLSLSPGK

SEQ ID NO: 194 - protein, 357 aa, synthetic construct
QLQLVESGGDLVQPGGSLRLSCLASGFTFSNHWMYWLRQAPGKGLEWVSDISPGGISTRYADSVKGRFTISRDNAKNTVYLEMSSLKPLDTAVYYCAAGRAYVAGVSRASQYVYWGQGTQVTVSSEPKSADKTHTCPPCPAPEAAGGPSVFLFPPKPKDTLMISRTPEVTCVVVDVSHEDPEVKFNWYVDGVEVHNAKTKPREEQYNSTYRVVSVLTVLHQDWLNGKEYKCKVSNKALPAPIEKTISKAKGQPREPQVYTLPPSREEMTKNQVSLTCLVKGFYPSDIAVEWESNGQPENNYKTTPPVLDSDGSFFLYSKLTVDKSRWQQGNVFSCSVMHEALHNHYTQKSLSLSPGK

SEQ ID NO: 195 - protein, 355 aa, synthetic construct
QLQLVESGGGLVQPGGSLRLSCAASGRTFSHYTVGWFRQAPGKEREFVAGLSWNHRTKYADSVKGRFTISVDNAKNTVYLQMNSLKPEDTAVYVCTADVSPFITTIQTDMEYWGKGTLVTVSSEPKSADKTHTCPPCPAPEAAGGPSVFLFPPKPKDTLMISRTPEVTCVVVDVSHEDPEVKFNWYVDGVEVHNAKTKPREEQYNSTYRVVSVLTVLHQDWLNGKEYKCKVSNKALPAPIEKTISKAKGQPREPQVYTLPPSREEMTKNQVSLTCLVKGFYPSDIAVEWESNGQPENNYKTTPPVLDSDGSFFLYSKLTVDKSRWQQGNVFSCSVMHEALHNHYTQKSLSLSPGK

SEQ ID NO: 196 - protein, 355 aa, synthetic construct
QLQLVESGGGLVQSGGSLRLSCTTSGIIFSKHGMGWYRQAPGAQRELVARITSGGSTSYADSGKGRFTISRDNTKNTLYLQMNSLEPEDTAVYYCNVERFIINVEGAGRGPYWGQGTLVTVSSEPKSADKTHTCPPCPAPEAAGGPSVFLFPPKPKDTLMISRTPEVTCVVVDVSHEDPEVKFNWYVDGVEVHNAKTKPREEQYNSTYRVVSVLTVLHQDWLNGKEYKCKVSNKALPAPIEKTISKAKGQPREPQVYTLPPSREEMTKNQVSLTCLVKGFYPSDIAVEWESNGQPENNYKTTPPVLDSDGSFFLYSKLTVDKSRWQQGNVFSCSVMHEALHNHYTQKSLSLSPGK

SEQ ID NO: 197 - protein, 357 aa, synthetic construct
QVQLVESGGGLVQAGGSLRLSCAVSGRTFSTLNMGWFRQAPGKEREFVANIGWSGGTTYSSDSAKGRFTISRDNAENTVYLQMNSLKPEDTAVYYCAADIKGLYFPRDARSFDYWGQGTQVTVSSEPKSADKTHTCPPCPAPEAAGGPSVFLFPPKPKDTLMISRTPEVTCVVVDVSHEDPEVKFNWYVDGVEVHNAKTKPREEQYNSTYRVVSVLTVLHQDWLNGKEYKCKVSNKALPAPIEKTISKAKGQPREPQVYTLPPSREEMTKNQVSLTCLVKGFYPSDIAVEWESNGQPENNYKTTPPVLDSDGSFFLYSKLTVDKSRWQQGNVFSCSVMHEALHNHYTQKSLSLSPGK

SEQ ID NO: 198 - protein, 355 aa, synthetic construct
QLQLVESGGGLVQAGGSLRLSCAASGRIFPIYHMGWFRQAPGKEREFVAAIRRSDSMTNYADSVKGRFTISRDNAKNTLFLQMNSLRPEDTGVYNCAAALGQYYGANTQYDSWGQGTQVTVSSEPKSADKTHTCPPCPAPEAAGGPSVFLFPPKPKDTLMISRTPEVTCVVVDVSHEDPEVKFNWYVDGVEVHNAKTKPREEQYNSTYRVVSVLTVLHQDWLNGKEYKCKVSNKALPAPIEKTISKAKGQPREPQVYTLPPSREEMTKNQVSLTCLVKGFYPSDIAVEWESNGQPENNYKTTPPVLDSDGSFFLYSKLTVDKSRWQQGNVFSCSVMHEALHNHYTQKSLSLSPGK

SEQ ID NO: 199 - protein, 351 aa, synthetic construct
QLQLVESGGGLVQPGGSLRLSCAASGSIFRFNLMGWYRQAPGKQRELVAVMSEGGTTNYGDSVKGRFTMSRDNAKNTVYLQMNSLKSEDTAVYYCNFWGSNSGPVLQYWGQGTQVTVSSEPKSADKTHTCPPCPAPEAAGGPSVFLFPPKPKDTLMISRTPEVTCVVVDVSHEDPEVKFNWYVDGVEVHNAKTKPREEQYNSTYRVVSVLTVLHQDWLNGKEYKCKVSNKALPAPIEKTISKAKGQPREPQVYTLPPSREEMTKNQVSLTCLVKGFYPSDIAVEWESNGQPENNYKTTPPVLDSDGSFFLYSKLTVDKSRWQQGNVFSCSVMHEALHNHYTQKSLSLSPGK

SEQ ID NO: 200 - protein, 356 aa, synthetic construct
QVQLVESGGGSVQPGGSLRLACAASGRIFVISNAGWFRQTPGKEREFVASISRHGEITNYADAVKGRFTISRDNSKNMMYLQMNSLNFEDTAVYYCATTLGHSPRTDPGDFDSWGQGTQVTVSSEPKSADKTHTCPPCPAPEAAGGPSVFLFPPKPKDTLMISRTPEVTCVVVDVSHEDPEVKFNWYVDGVEVHNAKTKPREEQYNSTYRVVSVLTVLHQDWLNGKEYKCKVSNKALPAPIEKTISKAKGQPREPQVYTLPPSREEMTKNQVSLTCLVKGFYPSDIAVEWESNGQPENNYKTTPPVLDSDGSFFLYSKLTVDKSRWQQGNVFSCSVMHEALHNHYTQKSLSLSPGK

SEQ ID NO: 201 - protein, 355 aa, synthetic construct
QVQLVESGGGLVQPGGSLRLSCAASGSIFRINTMGWYRQAPGKQRELVASFTSGGSPNYADSVKGRFTISRDNAKNTVYLQMNSLRPEETAVYYCNAYIMAWSHGVLKGYDSWGQGTQVTVSSEPKSADKTHTCPPCPAPEAAGGPSVFLFPPKPKDTLMISRTPEVTCVVVDVSHEDPEVKFNWYVDGVEVHNAKTKPREEQYNSTYRVVSVLTVLHQDWLNGKEYKCKVSNKALPAPIEKTISKAKGQPREPQVYTLPPSREEMTKNQVSLTCLVKGFYPSDIAVEWESNGQPENNYKTTPPVLDSDGSFFLYSKLTVDKSRWQQGNVFSCSVMHEALHNHYTQKSLSLSPGK

SEQ ID NO: 202 - protein, 353 aa, synthetic construct
QVQLVESGGGLVQPGESLRLSCAASGSIRTVNYMGWHRQAPGKQRELVAVVTSGGGTNYADSVKGRFTISRDDTKNTVYLAMNSLKPEDTAVYYCNAAASTYSSTVVRSFWGQGTQVTVSSEPKSADKTHTCPPCPAPEAAGGPSVFLFPPKPKDTLMISRTPEVTCVVVDVSHEDPEVKFNWYVDGVEVHNAKTKPREEQYNSTYRVVSVLTVLHQDWLNGKEYKCKVSNKALPAPIEKTISKAKGQPREPQVYTLPPSREEMTKNQVSLTCLVKGFYPSDIAVEWESNGQPENNYKTTPPVLDSDGSFFLYSKLTVDKSRWQQGNVFSCSVMHEALHNHYTQKSLSLSPGK

SEQ ID NO: 203 - protein, 356 aa, synthetic construct
QVQLVESGGGLVQPGGSLRLSCAASGSIFRINSMGWYRQAPGKQRELVATFTTSGGVTNYADSVKGRFTISRDNAKNTVYLQMNNLTPEETAVYYCNAYVMAWSRGVLKGYDSWGQGTQVTVSSEPKSADKTHTCPPCPAPEAAGGPSVFLFPPKPKDTLMISRTPEVTCVVVDVSHEDPEVKFNWYVDGVEVHNAKTKPREEQYNSTYRVVSVLTVLHQDWLNGKEYKCKVSNKALPAPIEKTISKAKGQPREPQVYTLPPSREEMTKNQVSLTCLVKGFYPSDIAVEWESNGQPENNYKTTPPVLDSDGSFFLYSKLTVDKSRWQQGNVFSCSVMHEALHNHYTQKSLSLSPGK

SEQ ID NO: 204 - protein, 355 aa, synthetic construct
QVQLVESGGGLVQAGGSLRLSCAASGRTFSGYRMGWFRQAPGKEREFVASIRWIGPATAYADSVKGRFTISRDNAKNTVYLQMNSLKSEDTAVYYCAADPTPSIDYKRGYDYWGQGTQVTVSSEPKSADKTHTCPPCPAPEAAGGPSVFLFPPKPKDTLMISRTPEVTCVVVDVSHEDPEVKFNWYVDGVEVHNAKTKPREEQYNSTYRVVSVLTVLHQDWLNGKEYKCKVSNKALPAPIEKTISKAKGQPREPQVYTLPPSREEMTKNQVSLTCLVKGFYPSDIAVEWESNGQPENNYKTTPPVLDSDGSFFLYSKLTVDKSRWQQGNVFSCSVMHEALHNHYTQKSLSLSPGK

SEQ ID NO: 205 - protein, 356 aa, synthetic construct
QVQLVESGGGLVQPGGSLRVSCAASGRTFNTFRTGWFRQAPGKEREFVASLNWSSTWTSYADSVKGRFSISRDSAKNTVYLQMNSLKPEDTADYYCAVGIAGTPVMRATSYIYWGQGTQVTVSSEPKSADKTHTCPPCPAPEAAGGPSVFLFPPKPKDTLMISRTPEVTCVVVDVSHEDPEVKFNWYVDGVEVHNAKTKPREEQYNSTYRVVSVLTVLHQDWLNGKEYKCKVSNKALPAPIEKTISKAKGQPREPQVYTLPPSREEMTKNQVSLTCLVKGFYPSDIAVEWESNGQPENNYKTTPPVLDSDGSFFLYSKLTVDKSRWQQGNVFSCSVMHEALHNHYTQKSLSLSPGK

SEQ ID NO: 206 - protein, 355 aa, synthetic construct
QVQLVESGGGLVQPGGSLRLSCAASRFIFPIYAMGWFRQAPGKEREFVAGIERTTDTTLYADSVKGRFTISRDNAKNTVYLQMYSLKPEDAAVYYCAARNSRRIGDVNDVDYWGQGTQVTVSSEPKSADKTHTCPPCPAPEAAGGPSVFLFPPKPKDTLMISRTPEVTCVVVDVSHEDPEVKFNWYVDGVEVHNAKTKPREEQYNSTYRVVSVLTVLHQDWLNGKEYKCKVSNKALPAPIEKTISKAKGQPREPQVYTLPPSREEMTKNQVSLTCLVKGFYPSDIAVEWESNGQPENNYKTTPPVLDSDGSFFLYSKLTVDKSRWQQGNVFSCSVMHEALHNHYTQKSLSLSPGK

SEQ ID NO: 207 - protein, 355 aa, synthetic construct
QLQLVESGGGLVQAGGSLRLSCAASRTIFPLYAMGWFRQAPGKEREFVAGISRTTSTTLYADSVKGRFTISRDNAANTVYLQMNTLKPEDAAVYYCAARNSRTIGDVNDVDYWGQGTQLTVSSEPKSADKTHTCPPCPAPEAAGGPSVFLFPPKPKDTLMISRTPEVTCVVVDVSHEDPEVKFNWYVDGVEVHNAKTKPREEQYNSTYRVVSVLTVLHQDWLNGKEYKCKVSNKALPAPIEKTISKAKGQPREPQVYTLPPSREEMTKNQVSLTCLVKGFYPSDIAVEWESNGQPENNYKTTPPVLDSDGSFFLYSKLTVDKSRWQQGNVFSCSVMHEALHNHYTQKSLSLSPGK

SEQ ID NO: 208 - protein, 356 aa, synthetic construct
QVQLVESGGGLVQAGGSLRLSCAASGRTISIYMMGWFRQAPGKGREFVSAIMPSGSRTYSADWVKGRFTISRDNSKSTVYLQMNSLKPEDTAVYYCAAKLFRGSGDYINDYDHWGQGTQVTVSSEPKSADKTHTCPPCPAPEAAGGPSVFLFPPKPKDTLMISRTPEVTCVVVDVSHEDPEVKFNWYVDGVEVHNAKTKPREEQYNSTYRVVSVLTVLHQDWLNGKEYKCKVSNKALPAPIEKTISKAKGQPREPQVYTLPPSREEMTKNQVSLTCLVKGFYPSDIAVEWESNGQPENNYKTTPPVLDSDGSFFLYSKLTVDKSRWQQGNVFSCSVMHEALHNHYTQKSLSLSPGK

SEQ ID NO: 209 - protein, 353 aa, synthetic construct
QVQLVESGGGLVQPGGSLRLSCAASGSIRTVNYMGWHRQAPGKQRELVAVVTSGGGTNYADSVKGRFTISRDDTKNTVYLQMNSLRAEDTAVYYCNAAASTYSSTVVRSFWGQGTLVTVSSEPKSADKTHTCPPCPAPEAAGGPSVFLFPPKPKDTLMISRTPEVTCVVVDVSHEDPEVKFNWYVDGVEVHNAKTKPREEQYNSTYRVVSVLTVLHQDWLNGKEYKCKVSNKALPAPIEKTISKAKGQPREPQVYTLPPSREEMTKNQVSLTCLVKGFYPSDIAVEWESNGQPENNYKTTPPVLDSDGSFFLYSKLTVDKSRWQQGNVFSCSVMHEALHNHYTQKSLSLSPGK

SEQ ID NO: 210 - protein, 353 aa, synthetic construct
QVQLVESGGGLVQPGGSLRLSCAASGSIRTVNYMGWHRQAPGKQRELVAVVTSGGGTNYADSVKGRFTISRDNTKNTVYLQMNSLRAEDTAVYYCNAAASTYSSTVVRSFWGQGTLVTVSSEPKSADKTHTCPPCPAPEAAGGPSVFLFPPKPKDTLMISRTPEVTCVVVDVSHEDPEVKFNWYVDGVEVHNAKTKPREEQYNSTYRVVSVLTVLHQDWLNGKEYKCKVSNKALPAPIEKTISKAKGQPREPQVYTLPPSREEMTKNQVSLTCLVKGFYPSDIAVEWESNGQPENNYKTTPPVLDSDGSFFLYSKLTVDKSRWQQGNVFSCSVMHEALHNHYTQKSLSLSPGK

SEQ ID NO: 211 - protein, 353 aa, synthetic construct
QVQLVESGGGLVQPGGSLRLSCAASGSIRTVNYMGWHRQAPGKQRELVAVVTSGGGTNYADSVKGRFTISRDDSKNTVYLQMNSLRAEDTAVYYCNAAASTYSSTVVRSFWGQGTLVTVSSEPKSADKTHTCPPCPAPEAAGGPSVFLFPPKPKDTLMISRTPEVTCVVVDVSHEDPEVKFNWYVDGVEVHNAKTKPREEQYNSTYRVVSVLTVLHQDWLNGKEYKCKVSNKALPAPIEKTISKAKGQPREPQVYTLPPSREEMTKNQVSLTCLVKGFYPSDIAVEWESNGQPENNYKTTPPVLDSDGSFFLYSKLTVDKSRWQQGNVFSCSVMHEALHNHYTQKSLSLSPGK

SEQ ID NO: 212 - protein, 353 aa, synthetic construct
QVQLVESGGGLVQPGGSLRLSCAASGSIRTVNYMGWHRQAPGKQRELVAVVTSGGGTNYADSVKGRFTISRDNSKNTVYLQMNSLRAEDTAVYYCNAAASTYSSTVVRSFWGQGTLVTVSSEPKSADKTHTCPPCPAPEAAGGPSVFLFPPKPKDTLMISRTPEVTCVVVDVSHEDPEVKFNWYVDGVEVHNAKTKPREEQYNSTYRVVSVLTVLHQDWLNGKEYKCKVSNKALPAPIEKTISKAKGQPREPQVYTLPPSREEMTKNQVSLTCLVKGFYPSDIAVEWESNGQPENNYKTTPPVLDSDGSFFLYSKLTVDKSRWQQGNVFSCSVMHEALHNHYTQKSLSLSPGK

SEQ ID NO: 213 - protein, 353 aa, synthetic construct
QVQLVESGGGLVQPGGSLRLSCAASGSIRTVNYMGWHRQAPGKGRELVAVVTSGGGTNYADSVKGRFTISRDDTKNTVYLQMNSLRAEDTAVYYCNAAASTYSSTVVRSFWGQGTLVTVSSEPKSADKTHTCPPCPAPEAAGGPSVFLFPPKPKDTLMISRTPEVTCVVVDVSHEDPEVKFNWYVDGVEVHNAKTKPREEQYNSTYRVVSVLTVLHQDWLNGKEYKCKVSNKALPAPIEKTISKAKGQPREPQVYTLPPSREEMTKNQVSLTCLVKGFYPSDIAVEWESNGQPENNYKTTPPVLDSDGSFFLYSKLTVDKSRWQQGNVFSCSVMHEALHNHYTQKSLSLSPGK

SEQ ID NO: 214 - protein, 353 aa, synthetic construct
QVQLVESGGGLVQPGGSLRLSCAASGSIRTVNYMGWHRQAPGKQLELVAVVTSGGGTNYADSVKGRFTISRDDTKNTVYLQMNSLRAEDTAVYYCNAAASTYSSTVVRSFWGQGTLVTVSSEPKSADKTHTCPPCPAPEAAGGPSVFLFPPKPKDTLMISRTPEVTCVVVDVSHEDPEVKFNWYVDGVEVHNAKTKPREEQYNSTYRVVSVLTVLHQDWLNGKEYKCKVSNKALPAPIEKTISKAKGQPREPQVYTLPPSREEMTKNQVSLTCLVKGFYPSDIAVEWESNGQPENNYKTTPPVLDSDGSFFLYSKLTVDKSRWQQGNVFSCSVMHEALHNHYTQKSLSLSPGK

SEQ ID NO: 215 - protein, 353 aa, synthetic construct
EVQLVESGGGLVQPGGSLRLSCAASGSIRTVNYMGWHRQAPGKQRELVAVVTSGGGTNYADSVKGRFTISRDDTKNTVYLQMNSLRAEDTAVYYCNAAASTYSSTVVRSFWGQGTLVTVSSEPKSADKTHTCPPCPAPEAAGGPSVFLFPPKPKDTLMISRTPEVTCVVVDVSHEDPEVKFNWYVDGVEVHNAKTKPREEQYNSTYRVVSVLTVLHQDWLNGKEYKCKVSNKALPAPIEKTISKAKGQPREPQVYTLPPSREEMTKNQVSLTCLVKGFYPSDIAVEWESNGQPENNYKTTPPVLDSDGSFFLYSKLTVDKSRWQQGNVFSCSVMHEALHNHYTQKSLSLSPGK

SEQ ID NO: 216 - protein, 353 aa, synthetic construct
QVQLVESGGGLVQPGGSLRLSCAASGSIRTVNYMGWHRQAPGKQRELVSVVTSGGGTNYADSVKGRFTISRDDTKNTVYLQMNSLRAEDTAVYYCNAAASTYSSTVVRSFWGQGTLVTVSSEPKSADKTHTCPPCPAPEAAGGPSVFLFPPKPKDTLMISRTPEVTCVVVDVSHEDPEVKFNWYVDGVEVHNAKTKPREEQYNSTYRVVSVLTVLHQDWLNGKEYKCKVSNKALPAPIEKTISKAKGQPREPQVYTLPPSREEMTKNQVSLTCLVKGFYPSDIAVEWESNGQPENNYKTTPPVLDSDGSFFLYSKLTVDKSRWQQGNVFSCSVMHEALHNHYTQKSLSLSPGK

SEQ ID NO: 217 - protein, 231 aa, synthetic construct
EPKSADKTHTCPPCPAPEAAGGPSVFLFPPKPKDTLYITREPEVTCVVVDVSHEDPEVKFNWYVDGVEVHNAKTKPREEQYNSTYRVVSVLTVLHQDWLNGKEYKCKVSNKALPAPIEKTISKAKGQPREPQVYTLPPSREEMTKNQVSLTCLVKGFYPSDIAVEWESNGQPENNYKTTPPVLDSDGSFFLYSKLTVDKSRWQQGNVFSCSVMHEALHNHYTQKSLSLSPG

SEQ ID NO: 218 - protein, 500 aa, synthetic construct
EVQLLESGGGLVQPGGSLRLSCAASGFTFGDYAITWFRQAPGKGLEGVAYISNFDGMTYYADSVKGRFTISSDNAKNTVYLQMNSLRAEDTAVYYCAAEGRMGTHSRDSVYFWAFSALYDYWGQGTLVTVSSEPKSADKTHTCPPCPAPEAAGGPSVFLFPPKPKDTLYITREPEVTCVVVDVSHEDPEVKFNWYVDGVEVHNAKTKPREEQYNSTYRVVSVLTVLHQDWLNGKEYKCKVSNKALPAPIEKTISKAKGQPREPQVYTLPPSREEMTKNQVSLTCLVKGFYPSDIAVEWESNGQPENNYKTTPPVLDSDGSFFLYSKLTVDKSRWQQGNVFSCSVMHEALHNHYTQKSLSLSPGGGGGSGGGGSGGGGSQVQLVESGGGLVQPGGSLRLSCAASGSIRTVNYMGWHRQAPGKQRELVAVVTSGGGTNYADSVKGRFTISRDNSKNTVYLQMNSLRAEDTAVYYCNAAASTYSSTVVRSFWGQGTLVTVSSA